European Patent Specification EP 3 630 825 B1, published February 14, 2024. Title: ANTI-HUMAN INTERLEUKIN-2 ANTIBODIES AND USES THEREOF. Applicant: INSTITUTE FOR BASIC SCIENCE POSTECH ACADEMY-INDUSTRY FOUNDATION. The sequence listing filed with the application follows.

SEQUENCE LISTING (34 sequences)

SEQ ID NO: 1 - DNA, 363 bp, Artificial Sequence
  TCB2 Heavy chain Variable region
gaggtgcaactgcagcagtctggggctgagctggcaagacctggggcttcagtgaagttgtcctgcaaggcttctggctacacctttactacctactggattcagtgggtgaaacagaggcctggacagggtctggaatggattggggctatttatcctggagatggtgatactaggtacattcagaatttcaagggcaaggccacattgactgcagataaatcctccagcacagcctacatgcaactcagcagcttggcatctgaggactctgcggtctattactgtgcaagatccctggcaactcggggcttctatgctatggactactggggtcaaggaacctcagtcaccgtctcctca

SEQ ID NO: 2 - DNA, 321 bp, Artificial Sequence
  TCB2 Light chain Variable region
gacattgtgatgacccagtctccagcatccctgtccatggctataggagaaaaagtcaccatcagatgcataaccagcactgatattgatgatgatatgaactggtaccagcagaagccaggggaacctcctaagctccttatttcagaaggcaatactcttcgtcctggagtcccatcccgattctccagcagtggctatggtacagattttgtttttacaattgaaaacatgctctcagaagatgttgcagattactactgtttgcaaagtgataacttgccgtacacgttcggaggggggaccaagctggaaataaaa

SEQ ID NO: 3 - protein, 120 aa, Artificial Sequence
  TCB2 Heavy chain Variable region
EVQLQQSGAELARPGASVKLSCKASGYTFTTYWIQWVKQRPGQGEWIGAIYPGDGDTRYIQNFKGKATLTADKSSSTAYMQLSSLASEDSAVYYCARSLATRGFYAMDYWGQGTSVTVSS

SEQ ID NO: 4 - protein, 107 aa, Artificial Sequence
  TCB2 Light chain Variable region
DIVMTQSPASLSMAIGEKVTIRCITSTDIDDDMNWYQQKPGEPPKLLISEGNTLRPGVPSRFSSSGYGTDFVFTIENMLSEDVADYYCLQSDNLPYTFGGGTKLEIK

SEQ ID NO: 5 - DNA, 15 bp, Artificial Sequence
  TCB2 Heavy chain CDR1
acctactggattcag

SEQ ID NO: 6 - DNA, 51 bp, Artificial Sequence
  TCB2 Heavy chain CDR2
gctatttatcctggagatggtgatactaggtacattcagaatttcaagggc

SEQ ID NO: 7 - DNA, 36 bp, Artificial Sequence
  TCB2 Heavy chain CDR3
tccctggcaactcggggcttctatgctatggactac

SEQ ID NO: 8 - DNA, 33 bp, Artificial Sequence
  TCB2 Light chain CDR1
ataaccagcactgatattgatgatgatatgaac

SEQ ID NO: 9 - DNA, 21 bp, Artificial Sequence
  TCB2 Light chain CDR2
gaaggcaatactcttcgtcct

SEQ ID NO: 10 - DNA, 27 bp, Artificial Sequence
  TCB2 Light chain CDR3
ttgcaaagtgataacttgccgtacacg

SEQ ID NO: 11 - protein, 5 aa, Artificial Sequence
  TCB2 Heavy chain CDR1
TYWIQ

SEQ ID NO: 12 - protein, 17 aa, Artificial Sequence
  TCB2 Heavy chain CDR2
AIYPGDGDTRYIQNFKG

SEQ ID NO: 13 - protein, 12 aa, Artificial Sequence
  TCB2 Heavy chain CDR3
SLATRGFYAMDY

SEQ ID NO: 14 - protein, 11 aa, Artificial Sequence
  TCB2 Light chain CDR1
ITSTDIDDDMN

SEQ ID NO: 15 - protein, 7 aa, Artificial Sequence
  TCB2 Light chain CDR2
EGNTLRP

SEQ ID NO: 16 - protein, 9 aa, Artificial Sequence
  TCB2 Light chain CDR3
LQSDNLPYT

SEQ ID NO: 17 - protein, 5 aa, Artificial Sequence
  Nara1 Heavy chain CDR1
NYLIE

SEQ ID NO: 18 - protein, 17 aa, Artificial Sequence
  Nara1 Heavy chain CDR2
VINPGSGGTNYNEKFKG

SEQ ID NO: 19 - protein, 12 aa, Artificial Sequence
  Nara1 Heavy chain CDR3
WRGDGYYAYFDV

SEQ ID NO: 20 - protein, 15 aa, Artificial Sequence
  Nara1 Light chain CDR1
KASQSVDYDGDSYMN

SEQ ID NO: 21 - protein, 7 aa, Artificial Sequence
  Nara1 Light chain CDR2
AASNLES

SEQ ID NO: 22 - protein, 9 aa, Artificial Sequence
  Nara1 Light chain CDR3
QQSNEDPYT

SEQ ID NO: 23 - protein, 447 aa, Artificial Sequence
  human chimeric TCB2 Heavy chain Variable region
EVQLQQSGAELARPGASVKLSCKASGYTFTTYWIQWVKQRPGQGLEWIGAIYPGDGDTRYIQNFKGKATLTADKSSSTAYMQLSSLASEDSAVYYCARSLATRGFYAMDYWGQGTSVTVSSASTKGPSVFPLAPCSRSTSESTAALGCLVKDYFPEPVTVSWNSGALTSGVHTFPAVLQSSGLYSLSSVVTVPSSNFGTQTYTCNVDHKPSNTKVDKTVERKCCVECPPCPAPPVAGPSVFLFPPKPKDTLMISRTPEVTCVVVDVSHEDPEVQFNWYVDGVEVHNAKTKPREEQFNSTFRVVSVLTVVHQDWLNGKEYKCKVSNKGLPAPIEKTISKTKGQPREPQVYTLPPSREEMTKNQVSLTCLVKGFYPSDIAVEWESNGQPENNYKTTPPMLDSDGSFFLYSKLTVDKSRWQQGNVFSCSVMHEALHNHYTQKSLSLSPGK

SEQ ID NO: 24 - protein, 214 aa, Artificial Sequence
  human chimeric TCB2 Light chain Variable region
DIVMTQSPASLSMAIGEKVTIRCITSTDIDDDMNWYQQKPGEPPKLLISEGNTLRPGVPSRFSSSGYGTDFVFTIENMLSEDVADYYCLQSDNLPYTFGGGTKLEIKRTVAAPSVFIFPPSDEQLKSGTASVVCLLNNFYPREAKVQWKVDNALQSGNSQESVTEQDSKDSTYSLSSTLTLSKADYEKHKVYACEVTHQGLSSPVTKSFNRGEC

SEQ ID NO: 25 - DNA, 321 bp, Artificial Sequence
  humanized TCB2_VL03463
gacattcagatgacccagagcccttccagcctgagcgccagcgtcggggacagagtgaccattacctgcattacctccacagacattgacgatgacatgaactggtaccagcagaagccagggaaagcccccaagctgctgatctatgagggaaatactctgcggcccggcgtgcctagcagattcagctcctctggctctgggaccgatttcacctttacaatcagttcactgcagcccgaagacattgctacatactattgcctgcagagcgacaacctgccttacaccttcgggggagggaccaaactggaaatcaaa

SEQ ID NO: 26 - protein, 107 aa, Artificial Sequence
  humanized TCB2_VL03463
DIQMTQSPSSLSASVGDRVTITCITSTDIDDDMNWYQQKPGKAPKLLIYEGNTLRPGVPSRFSSSGSGTDFTFTISSLQPEDIATYYCLQSDNLPYTFGGGTKLEIK

SEQ ID NO: 27 - DNA, 363 bp, Artificial Sequence
  humanized TCB2_VH03463
gaagtgcagctggtgcagagcggagcagaagtgaaaaagcctggggcaagcgtgaaggtgtcctgtaaagcaagcggatatacattcaccacatactggatccagtgggtgaagcaggcaccaggacagggactggagtggatgggagcaatctaccctggagacggcgatacacgatatattcagaacttcaaaggccgggtgactatgaccagagacacatctactagtaccgtctatatggagctgagctccctgaggagcgaagataccgctgtctactattgcgcccgctctctggctacaagagggttctacgctatggattattggggacaggggacactggtcaccgtcagcagc

SEQ ID NO: 28 - protein, 121 aa, Artificial Sequence
  humanized TCB2_VH03463
EVQLVQSGAEVKKPGASVKVSCKASGYTFTTYWIQWVKQAPGQGLEWMGAIYPGDGDTRYIQNFKGRVTMTRDTSTSTVYMELSSLRSEDTAVYYCARSLATRGFYAMDYWGQGTLVTVSS

SEQ ID NO: 29 - DNA, 321 bp, Artificial Sequence
  humanized TCB2_VL2
gacatcgtgatgacccagagccccagttccctgagcgccagcgtcggagacagagtgactattaggtgtattacttccacagatattgacgatgacatgaactggtaccagcagaagccaggcaaagcccccaagctgctgatcagcgagggaaatactctgcgaccaggagtgccttctagattctctggcagtgggtatggaaccgatttcacctttacaatcagctccctgcagcccgaagatattgctgactactattgcctgcagagcgataacctgccatacaccttcggcggggggaccaaactggaaatcaaa

SEQ ID NO: 30 - protein, 107 aa, Artificial Sequence
  humanized TCB2_VL2
DIVMTQSPSSLSASVGDRVTIRCITSTDIDDDMNWYQQKPGKAPKLLISEGNTLRPGVPSRFSGSGYGTDFTFTISSLQPEDIADYYCLQSDNLPYTFGGGTKLEIK

SEQ ID NO: 31 - DNA, 363 bp, Artificial Sequence
  humanized TCB2_VH1
caggtgcagctggtccagtcaggagcagaagtcaagaagcccggagcaagcgtcaaagtgtcatgcaaagcaagcggatatacatttaccacatactggatccagtgggtgcgacaggcaccaggacagggactggagtggatgggagcaatctaccctggagacggcgatacaagatatattcagaacttcaagggccgggtgactatgaccagagacacatctactagtaccgtctatatggagctgagctccctgaggagcgaagataccgctgtctactattgcgcccgctctctggctacaagggggttctacgcaatggattactgggggcaggggacactggtcaccgtctcatca

SEQ ID NO: 32 - protein, 121 aa, Artificial Sequence
  humanized TCB2_VH1
QVQLVQSGAEVKKPGASVKVSCKASGYTFTTYWIQWVRQAPGQGLEWMGAIYPGDGDTRYIQNFKGRVTMTRDTSTSTVYMELSSLRSEDTAVYYCARSLATRGFYAMDYWGQGTLVTVSS

SEQ ID NO: 33 - DNA, 363 bp, Artificial Sequence
  humanized TCB2_VH2
caggtccagctggtccagagcggagccgaggtgaagaagcccggagcaagcgtcaaactgtcatgcaaggcaagcggatacactttcaccacatactggatccagtgggtgaagcaggcaccaggacagggactggagtggatcggagcaatctaccctggagacggcgatacacggtatattcagaacttcaaaggcagagtgactatgaccgctgacacatctactagtaccgtctatatggagctgagctccctgaggagcgaagataccgccgtctactattgcgcccggtctctggctacaaggggcttttatgctatggattattggggacagggcacactggtcaccgtctcatct

SEQ ID NO: 34 - protein, 121 aa, Artificial Sequence
  humanized TCB2_VH2
QVQLVQSGAEVKKPGASVKLSCKASGYTFTTYWIQWVKQAPGQGLEWIGAIYPGDGDTRYIQNFKGRVTMTADTSTSTVYMELSSLRSEDTAVYYCARSLATRGFYAMDYWGQGTLVTVSS